European Patent Application EP 4 775 675 A1, published July 15, 2026. Title: 抗BDCA-2特异性抗体及其用途. Applicant: 上海宏成药业有限公司. The sequence listing filed with the application follows.

SEQUENCE LISTING (43 sequences)

SEQ ID NO: 1 - protein, 5 aa, synthetic construct
SYGMS

SEQ ID NO: 2 - protein, 17 aa, synthetic construct
TISSGDSYTYYPDSVKG

SEQ ID NO: 3 - protein, 12 aa, synthetic construct
QLYYSYGYYFDY

SEQ ID NO: 4 - protein, 15 aa, synthetic construct
RASESVSFHGTHLMH

SEQ ID NO: 5 - protein, 7 aa, synthetic construct
AASNLES

SEQ ID NO: 6 - protein, 9 aa, synthetic construct
QQSIEDPPT

SEQ ID NO: 7 - protein, 121 aa, synthetic construct
EVQLVESGGDLVKPGGSLKLSCAASGFTFSSYGMSWVRQTPDKRLEWVATISSGDSYTYYPDSVKGRFTISRDNAKNTLYLQMSSLKSEDTAMYYCARQLYYSYGYYFDYWGQGTTLTVSS

SEQ ID NO: 8 - protein, 111 aa, synthetic construct
DIVLTQSPASLAVSLGQRATISCRASESVSFHGTHLMHWYQQKPGQPPKLLIYAASNLESGVPARFSGSGSETDFTLNIHPVEEEDAATYFCQQSIEDPPTFGGGTKLEIK

SEQ ID NO: 9 - protein, 330 aa, synthetic construct [sequence omitted]

SEQ ID NO: 10 - protein, 107 aa, synthetic construct [sequence omitted]

SEQ ID NO: 11 - protein, 5 aa, synthetic construct
TYTMS

SEQ ID NO: 12 - protein, 17 aa, synthetic construct
TINSGGDNTYYPDSVKG

SEQ ID NO: 13 - protein, 12 aa, synthetic construct
YRPYYYGSVLDY

SEQ ID NO: 14 - protein, 15 aa, synthetic construct
KASQSVDYDGNSYVN

SEQ ID NO: 15 - protein, 7 aa, synthetic construct
GASNLES

SEQ ID NO: 16 - protein, 9 aa, synthetic construct
QQSDEDPWT

SEQ ID NO: 17 - protein, 121 aa, synthetic construct
DVILVESGGGLVKPGGSLKLSCAASGITFSTYTMSWLRQTPEKRLEWVATINSGGDNTYYPDSVKGRFTISRDNAKNNLYLQMSSLKSEDTALYYCATYRPYYYGSVLDYWGQGTTLTVSS

SEQ ID NO: 18 - protein, 111 aa, synthetic construct
DIVLTQSPASLAVSLGQRATISCKASQSVDYDGNSYVNWYQQKPGQPPKLLIYGASNLESGIPDRFSGSGSGTDFTLNIHPVEEEDGATYYCQQSDEDPWTFGGGTKLEIR

SEQ ID NO: 19 - protein, 121 aa, synthetic construct
EVQLVESGGGLVKPGGSLRLSCAASGFTFSSYGMSWVRQAPGKGLEWVSTISSGDSYTYYPDSVKGRFTISRDNAKNSLYLQMNSLRAEDTAVYYCARQLYYSYGYYFDYWGQGTTVTVSS

SEQ ID NO: 20 - protein, 121 aa, synthetic construct
EVQLVESGGGLVKPGGSLRLSCAASGFTFSSYGMSWVRQAPGKGLEWVATISSGDSYTYYPDSVKGRFTISRDNAKNSLYLQMNSLRAEDTAVYYCARQLYYSYGYYFDYWGQGTTVTVSS

SEQ ID NO: 21 - protein, 121 aa, synthetic construct
EVQLVESGGGLVKPGGSLRLSCAASGFTFSSYGMSWVRQAPGKRLEWVATISSGDSYTYYPDSVKGRFTISRDNAKNSLYLQMNSLRAEDTAVYYCARQLYYSYGYYFDYWGQGTTVTVSS

SEQ ID NO: 22 - protein, 111 aa, synthetic construct
DIVLTQSPASLAVSPGQRATITCRASESVSFHGTHLMHWYQQKPGQPPKLLIYAASNLESGVPARFSGSGSGTDFTLTINPVEAEDTANYYCQQSIEDPPTFGGGTKVEIK

SEQ ID NO: 23 - protein, 111 aa, synthetic construct
DIVLTQSPASLAVSPGQRATITCRASESVSFHGTHLMHWYQQKPGQPPKLLIYAASNLESGVPARFSGSGSGTDFTLTINPVEANDAANYYCQQSIEDPPTFGGGTKVEIK

SEQ ID NO: 24 - protein, 111 aa, synthetic construct
DIVLTQSPASLAVSPGQRATITCRASESVSFHGTHLMHWYQQKPGQPPKLLIYAASNLESGVPARFSGSGSETDFTLTINPVEAEDTANYYCQQSIEDPPTFGGGTKVEIK

SEQ ID NO: 25 - protein, 111 aa, synthetic construct
DIVLTQSPASLAVSPGQRATITCRASESVSFHGTHLMHWYQQKPGQPPKLLIYAASNLESGVPARFSGSGSETDFTLTINPVEANDAANYYCQQSIEDPPTFGGGTKVEIK

SEQ ID NO: 26 - protein, 121 aa, synthetic construct
EVQLLESGGGLVQPGGSLRLSCAASGFTFSTYTMSWVRQAPGKGLEWVSTINSGGDNTYYPDSVKGRFTISRDNSKNTLYLQMNSLRAEDTAVYYCATYRPYYYGSVLDYWGQGTTVTVSS

SEQ ID NO: 27 - protein, 121 aa, synthetic construct
EVQLLESGGGLVQPGGSLRLSCAASGFTFSTYTMSWVRQAPGKGLEWVATINSGGDNTYYPDSVKGRFTISRDNSKNTLYLQMNSLRAEDTAVYYCATYRPYYYGSVLDYWGQGTTVTVSS

SEQ ID NO: 28 - protein, 121 aa, synthetic construct
EVQLLESGGGLVQPGGSLRLSCAASGITFSTYTMSWVRQAPGKGLEWVATINSGGDNTYYPDSVKGRFTISRDNSKNTLYLQMNSLRAEDTAVYYCATYRPYYYGSVLDYWGQGTTVTVSS

SEQ ID NO: 29 - protein, 121 aa, synthetic construct
EVQLLESGGGLVQPGGSLRLSCAASGITFSTYTMSWVRQAPGKRLEWVATINSGGDNTYYPDSVKGRFTISRDNSKNTLYLQMNSLRAEDTAVYYCATYRPYYYGSVLDYWGQGTTVTVSS

SEQ ID NO: 30 - protein, 111 aa, synthetic construct
DIVMTQSPDSLAVSLGERATINCKASQSVDYDGNSYVNWYQQKPGQPPKLLIYGASNLESGVPDRFSGSGSGTDFTLTISSLQAEDVAVYYCQQSDEDPWTFGGGTKVEIK

SEQ ID NO: 31 - protein, 111 aa, synthetic construct
DIVMTQSPDSLAVSLGERATINCKASQSVDYDGNSYVNWYQQKPGQPPKLLIYGASNLESGIPDRFSGSGSGTDFTLTISSLQAEDVAVYYCQQSDEDPWTFGGGTKVEIK

SEQ ID NO: 32 - protein, 111 aa, synthetic construct
DIVLTQSPDSLAVSLGERATINCKASQSVDYDGNSYVNWYQQKPGQPPKLLIYGASNLESGIPDRFSGSGSGTDFTLTISSLQAEDVAVYYCQQSDEDPWTFGGGTKVEIK

SEQ ID NO: 33 - protein, 451 aa, synthetic construct
EVQLVESGGDLVKPGGSLKLSCAASGFTFSSYGMSWVRQTPDKRLEWVATISSGDSYTYYPDSVKGRFTISRDNAKNTLYLQMSSLKSEDTAMYYCARQLYYSYGYYFDYWGQGTTLTVSSASTKGPSVFPLAPSSKSTSGGTAALGCLVKDYFPEPVTVSWNSGALTSGVHTFPAVLQSSGLYSLSSVVTVPSSSLGTQTYICNVNHKPSNTKVDKKVEPKSCDKTHTCPPCPAPELLGGPSVFLFPPKPKDTLMISRTPEVTCVVVDVSHEDPEVKFNWYVDGVEVHNAKTKPREEQYNSTYRVVSVLTVLHQDWLNGKEYKCKVSNKALPAPIEKTISKAKGQPREPQVYTLPPSRDELTKNQVSLTCLVKGFYPSDIAVEWESNGQPENNYKTTPPVLDSDGSFFLYSKLTVDKSRWQQGNVFSCSVMHEALHNHYTQKSLSLSPGK

SEQ ID NO: 34 - protein, 218 aa, synthetic construct
DIVLTQSPASLAVSLGQRATISCRASESVSFHGTHLMHWYQQKPGQPPKLLIYAASNLESGVPARFSGSGSETDFTLNIHPVEEEDAATYFCQQSIEDPPTFGGGTKLEIKRTVAAPSVFIFPPSDEQLKSGTASVVCLLNNFYPREAKVQWKVDNALQSGNSQESVTEQDSKDSTYSLSSTLTLSKADYEKHKVYACEVTHQGLSSPVTKSFNRGEC

SEQ ID NO: 35 - protein, 451 aa, synthetic construct
DVILVESGGGLVKPGGSLKLSCAASGITFSTYTMSWLRQTPEKRLEWVATINSGGDNTYYPDSVKGRFTISRDNAKNNLYLQMSSLKSEDTALYYCATYRPYYYGSVLDYWGQGTTLTVSSASTKGPSVFPLAPSSKSTSGGTAALGCLVKDYFPEPVTVSWNSGALTSGVHTFPAVLQSSGLYSLSSVVTVPSSSLGTQTYICNVNHKPSNTKVDKKVEPKSCDKTHTCPPCPAPELLGGPSVFLFPPKPKDTLMISRTPEVTCVVVDVSHEDPEVKFNWYVDGVEVHNAKTKPREEQYNSTYRVVSVLTVLHQDWLNGKEYKCKVSNKALPAPIEKTISKAKGQPREPQVYTLPPSRDELTKNQVSLTCLVKGFYPSDIAVEWESNGQPENNYKTTPPVLDSDGSFFLYSKLTVDKSRWQQGNVFSCSVMHEALHNHYTQKSLSLSPGK

SEQ ID NO: 36 - protein, 218 aa, synthetic construct
DIVLTQSPASLAVSLGQRATISCKASQSVDYDGNSYVNWYQQKPGQPPKLLIYGASNLESGIPDRFSGSGSGTDFTLNIHPVEEEDGATYYCQQSDEDPWTFGGGTKLEIRRTVAAPSVFIFPPSDEQLKSGTASVVCLLNNFYPREAKVQWKVDNALQSGNSQESVTEQDSKDSTYSLSSTLTLSKADYEKHKVYACEVTHQGLSSPVTKSFNRGEC

SEQ ID NO: 37 - protein, 451 aa, synthetic construct
EVQLVESGGGLVKPGGSLRLSCAASGFTFSSYGMSWVRQAPGKGLEWVSTISSGDSYTYYPDSVKGRFTISRDNAKNSLYLQMNSLRAEDTAVYYCARQLYYSYGYYFDYWGQGTTVTVSSASTKGPSVFPLAPSSKSTSGGTAALGCLVKDYFPEPVTVSWNSGALTSGVHTFPAVLQSSGLYSLSSVVTVPSSSLGTQTYICNVNHKPSNTKVDKKVEPKSCDKTHTCPPCPAPELLGGPSVFLFPPKPKDTLMISRTPEVTCVVVDVSHEDPEVKFNWYVDGVEVHNAKTKPREEQYNSTYRVVSVLTVLHQDWLNGKEYKCKVSNKALPAPIEKTISKAKGQPREPQVYTLPPSRDELTKNQVSLTCLVKGFYPSDIAVEWESNGQPENNYKTTPPVLDSDGSFFLYSKLTVDKSRWQQGNVFSCSVMHEALHNHYTQKSLSLSPGK

SEQ ID NO: 38 - protein, 218 aa, synthetic construct
DIVLTQSPASLAVSPGQRATITCRASESVSFHGTHLMHWYQQKPGQPPKLLIYAASNLESGVPARFSGSGSGTDFTLTINPVEAEDTANYYCQQSIEDPPTFGGGTKVEIKRTVAAPSVFIFPPSDEQLKSGTASVVCLLNNFYPREAKVQWKVDNALQSGNSQESVTEQDSKDSTYSLSSTLTLSKADYEKHKVYACEVTHQGLSSPVTKSFNRGEC

SEQ ID NO: 39 - protein, 218 aa, synthetic construct
DIVLTQSPASLAVSPGQRATITCRASESVSFHGTHLMHWYQQKPGQPPKLLIYAASNLESGVPARFSGSGSGTDFTLTINPVEANDAANYYCQQSIEDPPTFGGGTKVEIKRTVAAPSVFIFPPSDEQLKSGTASVVCLLNNFYPREAKVQWKVDNALQSGNSQESVTEQDSKDSTYSLSSTLTLSKADYEKHKVYACEVTHQGLSSPVTKSFNRGEC

SEQ ID NO: 40 - protein, 218 aa, synthetic construct
DIVLTQSPASLAVSPGQRATITCRASESVSFHGTHLMHWYQQKPGQPPKLLIYAASNLESGVPARFSGSGSETDFTLTINPVEAEDTANYYCQQSIEDPPTFGGGTKVEIKRTVAAPSVFIFPPSDEQLKSGTASVVCLLNNFYPREAKVQWKVDNALQSGNSQESVTEQDSKDSTYSLSSTLTLSKADYEKHKVYACEVTHQGLSSPVTKSFNRGEC

SEQ ID NO: 41 - protein, 218 aa, synthetic construct
DIVLTQSPASLAVSPGQRATITCRASESVSFHGTHLMHWYQQKPGQPPKLLIYAASNLESGVPARFSGSGSETDFTLTINPVEANDAANYYCQQSIEDPPTFGGGTKVEIKRTVAAPSVFIFPPSDEQLKSGTASVVCLLNNFYPREAKVQWKVDNALQSGNSQESVTEQDSKDSTYSLSSTLTLSKADYEKHKVYACEVTHQGLSSPVTKSFNRGEC

SEQ ID NO: 42 - protein, 451 aa, synthetic construct
EVQLVESGGGLVKPGGSLRLSCAASGFTFSSYGMSWVRQAPGKGLEWVATISSGDSYTYYPDSVKGRFTISRDNAKNSLYLQMNSLRAEDTAVYYCARQLYYSYGYYFDYWGQGTTVTVSSASTKGPSVFPLAPSSKSTSGGTAALGCLVKDYFPEPVTVSWNSGALTSGVHTFPAVLQSSGLYSLSSVVTVPSSSLGTQTYICNVNHKPSNTKVDKKVEPKSCDKTHTCPPCPAPELLGGPSVFLFPPKPKDTLMISRTPEVTCVVVDVSHEDPEVKFNWYVDGVEVHNAKTKPREEQYNSTYRVVSVLTVLHQDWLNGKEYKCKVSNKALPAPIEKTISKAKGQPREPQVYTLPPSRDELTKNQVSLTCLVKGFYPSDIAVEWESNGQPENNYKTTPPVLDSDGSFFLYSKLTVDKSRWQQGNVFSCSVMHEALHNHYTQKSLSLSPGK

SEQ ID NO: 43 - protein, 451 aa, synthetic construct
EVQLVESGGGLVKPGGSLRLSCAASGFTFSSYGMSWVRQAPGKRLEWVATISSGDSYTYYPDSVKGRFTISRDNAKNSLYLQMNSLRAEDTAVYYCARQLYYSYGYYFDYWGQGTTVTVSSASTKGPSVFPLAPSSKSTSGGTAALGCLVKDYFPEPVTVSWNSGALTSGVHTFPAVLQSSGLYSLSSVVTVPSSSLGTQTYICNVNHKPSNTKVDKKVEPKSCDKTHTCPPCPAPELLGGPSVFLFPPKPKDTLMISRTPEVTCVVVDVSHEDPEVKFNWYVDGVEVHNAKTKPREEQYNSTYRVVSVLTVLHQDWLNGKEYKCKVSNKALPAPIEKTISKAKGQPREPQVYTLPPSRDELTKNQVSLTCLVKGFYPSDIAVEWESNGQPENNYKTTPPVLDSDGSFFLYSKLTVDKSRWQQGNVFSCSVMHEALHNHYTQKSLSLSPGK